European Patent Specification EP 3 464 612 B1, published October 30, 2024. Title: TWO-COLOR NANOPORE SEQUENCING. Applicant: Quantapore, Inc. Guegler, Karl Simons, Jan Macevicz, Stephen. The sequence listing filed with the application follows.

SEQUENCE LISTING (2 sequences)

SEQ ID NO: 1 - DNA, 25 bp, Artificial Sequence
  random sequence
accgtttaaaggtttccccgtcgta

SEQ ID NO: 2 - RNA, 44 nt, Artificial Sequence
  random sequence
accguuuaaagguuuccccgucguaaaaaaaaaaaaaaaaaaaa